European Patent Application EP 4 471 123 A1, published December 4, 2024. Title: METHOD FOR CONSTRUCTING THREONINE-PRODUCING ENGINEERED BACTERIUM. Applicant: Langfang Meihua Biotechnology Development Co.,Ltd. Application EP 22923646.8, filed December 29, 2022. The sequence listing filed with the application follows.

SEQUENCE LISTING (46 sequences)

SEQ ID NO: 1 - DNA, 1266 bp, Corynebacterium glutamicum
  source 1..1266: mol_type = genomic DNA
gtggccctggtcgtacagaaatatggcggttcctcgcttgagagtgcggaacgcattagaaacgtcgctgaacggatcgttgccaccaagaaggctggaaatgatgtcgtggttgtctgctccgcaatgggagacaccacggatgaacttctagaacttgcagcggcagtgaatcccgttccgccagctcgtgaaatggatatgctcctgactgctggtgagcgtatttctaacgctctcgtcgccatggctattgagtcccttggcgcagaagcccaatctttcacgggctctcaggctggtgtgctcaccaccgagcgccacggaaacgcacgcattgttgatgtcactccaggtcgtgtgcgtgaagcactcgatgagggcaagatctgcattgttgctggtttccagggtgttaataaagaaacccgcgatgtcaccacgttgggtcgtggtggttctgacaccactgcagttgcgttggcagctgctttgaacgctgatgtgtgtgagatttactcggacgttgacggtgtgtataccgctgacccgcgcatcgttcctaatgcacagaagctggaaaagctcagcttcgaagaaatgctggaacttgctgctgttggctccaagattttggtgctgcgcagtgttgaatacgctcgtgcattcaatgtgccacttcgcgtacgctcgtcttatagtaatgatcccggcactttgattgccggctctatggaggatattcctgtggaagaagcagtccttaccggtgtcgcaaccgacaagtccgaagccaaagtaaccgttctgggtatttccgataagccaggcgaggctgcgaaggttttccgtgcgttggctgatgcagaaatcaacattgacatggttctgcagaacgtctcttctgtagaagacggcaccaccgacatcaccttcacctgccctcgttccgacggccgccgcgcgatggagatcttgaagaagcttcaggttcagggcaactggaccaatgtgctttacgacgaccaggtcggcaaagtctccctcgtgggtgctggcatgaagtctcacccaggtgttaccgcagagttcatggaagctctgcgcgatgtcaacgtgaacatcgaattgatttccacctctgagattcgtatttccgtgctgatccgtgaagatgatctggatgctgctgcacgtgcattgcatgagcagttccagctgggcggcgaagacgaagccgtcgtttatgcaggcaccggacgctaa

SEQ ID NO: 2 - DNA, 1446 bp, Corynebacterium glutamicum
  source 1..1446: mol_type = genomic DNA
gtggactacatttcgacgcgtgatgccagccgtacccctgcccgcttcagtgatattttgctgggcggtctagcaccagacggcggcctgtacctgcctgcaacctaccctcaactagatgatgcccagctgagtaaatggcgtgaggtattagccaacgaaggatacgcagctttggctgctgaagttatctccctgtttgttgatgacatcccagtagaagacatcaaggcgatcaccgcacgcgcctacacctacccgaagttcaacagcgaagacatcgttcctgtcaccgaactcgaggacaacatttacctgggccacctttccgaaggcccaaccgctgcattcaaagacatggccatgcagctgctcggcgaacttttcgaatacgagcttcgccgccgcaacgaaaccatcaacatcctgggcgctacctctggcgataccggctcctctgcggaatacgccatgcgcggccgcgagggaatccgcgtattcatgctgaccccagctggccgcatgaccccattccagcaagcacagatgtttggccttgacgatccaaacatcttcaacatcgccctcgacggcgttttcgacgattgccaagacgtagtcaaggctgtctccgccgacgcagaattcaaaaaagacaaccgcatcggtgccgtgaactccatcaactgggcacgccttatggcacaggttgtgtactacgtttcctcatggatccgcaccacaaccagcaatgaccaaaaggtcagcttctccgtaccaaccggcaacttcggtgacatttgcgcaggccacatcgcccgccaaatgggacttcccatcgatcgcctcatcgtggccaccaacgaaaacgatgtgctcgacgagttcttccgtaccggcgactaccgagtccgcagctccgcagacacccacgagacctcctcaccttcgatggatatctcccgcgcctccaacttcgagcgtttcatcttcgacctgctcggccgcgacgccacccgcgtcaacgatctatttggtacccaggttcgccaaggcggattctcactggctgatgacgccaactttgagaaggctgcagcagaatacggtttcgcctccggacgatccacccatgctgaccgtgtggcaaccatcgctgacgtgcattcccgcctcgacgtactaatcgatccccacaccgccgacggcgttcacgtggcacgccagtggagggacgaggtcaacaccccaatcatcgtcctagaaactgcactcccagtgaaatttgccgacaccatcgtcgaagcaattggtgaagcacctcaaactccagagcgtttcgccgcgatcatggatgctccattcaaggtttccgacctaccaaacgacaccgatgcagttaagcagtacatagtcgatgcgattgcaaacacttccgtgaagtaa

SEQ ID NO: 3 - DNA, 46 bp, synthetic construct
  source 1..46: mol_type = other DNA
aattcgagctcggtacccggggatccagcgacaggacaagcactgg

SEQ ID NO: 4 - DNA, 40 bp, synthetic construct
  source 1..40: mol_type = other DNA
cccggaataattggcagctatgtgcacctttcgatctacg

SEQ ID NO: 5 - DNA, 40 bp, synthetic construct
  source 1..40: mol_type = other DNA
cgtagatcgaaaggtgcacatagctgccaattattccggg

SEQ ID NO: 6 - DNA, 41 bp, synthetic construct
  source 1..41: mol_type = other DNA
tttctgtacgaccagggccatgggtaaaaaatcctttcgta

SEQ ID NO: 7 - DNA, 41 bp, synthetic construct
  source 1..41: mol_type = other DNA
tacgaaaggattttttacccatggccctggtcgtacagaaa

SEQ ID NO: 8 - DNA, 42 bp, synthetic construct
  source 1..42: mol_type = other DNA
tcggaacgagggcaggtgaaggtgatgtcggtggtgccgtct

SEQ ID NO: 9 - DNA, 42 bp, synthetic construct
  source 1..42: mol_type = other DNA
agacggcaccaccgacatcaccttcacctgccctcgttccga

SEQ ID NO: 10 - DNA, 46 bp, synthetic construct
  source 1..46: mol_type = other DNA
gtaaaacgacggccagtgccaagcttagcctggtaagaggaaacgt

SEQ ID NO: 11 - DNA, 46 bp, synthetic construct
  source 1..46: mol_type = other DNA
aattcgagctcggtacccggggatccctgcgggcagatccttttga

SEQ ID NO: 12 - DNA, 40 bp, synthetic construct
  source 1..40: mol_type = other DNA
atttctttataaacgcaggtcatatctaccaaaactacgc

SEQ ID NO: 13 - DNA, 40 bp, synthetic construct
  source 1..40: mol_type = other DNA
gcgtagttttggtagatatgacctgcgtttataaagaaat

SEQ ID NO: 14 - DNA, 40 bp, synthetic construct
  source 1..40: mol_type = other DNA
gtatatctccttctgcaggaataggtatcgaaagacgaaa

SEQ ID NO: 15 - DNA, 40 bp, synthetic construct
  source 1..40: mol_type = other DNA
tttcgtctttcgatacctattcctgcagaaggagatatac

SEQ ID NO: 16 - DNA, 41 bp, synthetic construct
  source 1..41: mol_type = other DNA
tagccaattcagccaaaacccccacgcgatcttccacatcc

SEQ ID NO: 17 - DNA, 41 bp, synthetic construct
  source 1..41: mol_type = other DNA
ggatgtggaagatcgcgtgggggttttggctgaattggcta

SEQ ID NO: 18 - DNA, 46 bp, synthetic construct
  source 1..46: mol_type = other DNA
gtaaaacgacggccagtgccaagcttgctggctcttgccgtcgata

SEQ ID NO: 19 - DNA, 46 bp, synthetic construct
  source 1..46: mol_type = other DNA
attcgagctcggtacccggggatccgccgttgatcattgttcttca

SEQ ID NO: 20 - DNA, 40 bp, synthetic construct
  source 1..40: mol_type = other DNA
cccggaataattggcagctaggatataaccctatcccaag

SEQ ID NO: 21 - DNA, 40 bp, synthetic construct
  source 1..40: mol_type = other DNA
cttgggatagggttatatcctagctgccaattattccggg

SEQ ID NO: 22 - DNA, 41 bp, synthetic construct
  source 1..41: mol_type = other DNA
acgcgtcgaaatgtagtccatgggtaaaaaatcctttcgta

SEQ ID NO: 23 - DNA, 41 bp, synthetic construct
  source 1..41: mol_type = other DNA
tacgaaaggattttttacccatggactacatttcgacgcgt

SEQ ID NO: 24 - DNA, 46 bp, synthetic construct
  source 1..46: mol_type = other DNA
gtaaaacgacggccagtgccaagcttgaatacgcggattccctcgc

SEQ ID NO: 25 - DNA, 46 bp, synthetic construct
  source 1..46: mol_type = other DNA
aattcgagctcggtacccggggatcctcatctgcggtgacatatcc

SEQ ID NO: 26 - DNA, 40 bp, synthetic construct
  source 1..40: mol_type = other DNA
cattcgcagggtaacggccactgaagggcctcctggggca

SEQ ID NO: 27 - DNA, 40 bp, synthetic construct
  source 1..40: mol_type = other DNA
tgccccaggaggcccttcagtggccgttaccctgcgaatg

SEQ ID NO: 28 - DNA, 40 bp, synthetic construct
  source 1..40: mol_type = other DNA
tcggggttctttaggttcattgtatgtcctcctggacttc

SEQ ID NO: 29 - DNA, 40 bp, synthetic construct
  source 1..40: mol_type = other DNA
gaagtccaggaggacatacaatgaacctaaagaaccccga

SEQ ID NO: 30 - DNA, 46 bp, synthetic construct
  source 1..46: mol_type = other DNA
gtaaaacgacggccagtgccaagcttgtgacgtcggaagggttgat

SEQ ID NO: 31 - DNA, 42 bp, synthetic construct
  source 1..42: mol_type = other DNA
gagctcggtacccggggatccgcagggtattgcagggactca

SEQ ID NO: 32 - DNA, 49 bp, synthetic construct
  source 1..49: mol_type = other DNA
caagcccggaataattggcagctaaactgcgtacctccgcatgtggtgg

SEQ ID NO: 33 - DNA, 25 bp, synthetic construct
  source 1..25: mol_type = other DNA
tagctgccaattattccgggcttgt

SEQ ID NO: 34 - DNA, 25 bp, synthetic construct
  source 1..25: mol_type = other DNA
gggtaaaaaatcctttcgtaggttt

SEQ ID NO: 35 - DNA, 53 bp, synthetic construct
  source 1..53: mol_type = other DNA
ggaaacctacgaaaggattttttacccatgagttcagtttcgctgcaggattt

SEQ ID NO: 36 - DNA, 41 bp, synthetic construct
  source 1..41: mol_type = other DNA
acgacggccagtgccaagcttacaccggaacaacccacatg

SEQ ID NO: 37 - DNA, 44 bp, synthetic construct
  source 1..44: mol_type = other DNA
gagctcggtacccggggatccgaagcgtctgaagtagtggcagt

SEQ ID NO: 38 - DNA, 45 bp, synthetic construct
  source 1..45: mol_type = other DNA
acattcgcagggtaacggccattattgcggaccttcctttacagc

SEQ ID NO: 39 - DNA, 25 bp, synthetic construct
  source 1..25: mol_type = other DNA
tggccgttaccctgcgaatgtccac

SEQ ID NO: 40 - DNA, 24 bp, synthetic construct
  source 1..24: mol_type = other DNA
tgtatgtcctcctggacttcgtgg

SEQ ID NO: 41 - DNA, 52 bp, synthetic construct
  source 1..52: mol_type = other DNA
caccacgaagtccaggaggacatacaatgactgcacccacgaacgctgggga

SEQ ID NO: 42 - DNA, 40 bp, synthetic construct
  source 1..40: mol_type = other DNA
acgacggccagtgccaagcttgcatcgagcactcccctgc

SEQ ID NO: 43 - DNA, 46 bp, synthetic construct
  source 1..46: mol_type = other DNA
aattcgagctcggtacccggggatccacgtgatggttcgacgcatc

SEQ ID NO: 44 - DNA, 40 bp, synthetic construct
  source 1..40: mol_type = other DNA
aaatcagcctcactgattagtcactcattgttttctcctt

SEQ ID NO: 45 - DNA, 40 bp, synthetic construct
  source 1..40: mol_type = other DNA
aaggagaaaacaatgagtgactaatcagtgaggctgattt

SEQ ID NO: 46 - DNA, 40 bp, synthetic construct
  source 1..40: mol_type = other DNA
gtaaaacgacggccagtgccaagctttggttgtcggatct